European Patent Specification EP 3 944 855 B1, published February 26, 2025. Title: Method for Screening of unpleasant odor masking agents. Applicant: Takasago International Corporation. The sequence listing filed with the application follows.

SEQUENCE LISTING (4 sequences)

SEQ ID NO: 1 - DNA, 939 bp, Homo sapiens
  CDS (1)..(939)
atggaaaattacaatcaaacatcaactgatttcatcttattaggattcttcccaccatcaagaattggccttttcctcttcatcctcattgttttcattttcctaatggctctaattggaaacctatccatgattcttctcatcttcttggacacccatctccacacacccatgtatttcctacttagtcagctctccctcattgacctaaattacatctccaccattgttcctaagatggcatctgattttctgtctggtaacaagtctatctccttcactgggtgtgggattcagagtttcttcttctcggcattaggaggtgcagaagcactacttttggcatctatggcctatgatcgttacattgctatttgctttcctcttcactatcccatccgcatgagcaaaagaatgtgtgtgctgatgataacagggtcttggatcataggctcgatcaatgcttgtgctcacactgtatatgtactccatattccttattgccaatccagggccatcaatcatttcttctgtgatgtcccagcaatggtgactctggcctgcatggacacctgggtctatgagggcacagtgtttttgagcaccaccatctttctcgtgtttcccttcattgctatttcatgttcctatggccgggttctccttgctgtctaccacatgaaatctgcagaagggaggaagaaagcctacctgacctgcagcacccacctcactgtagtaactttctactatgcaccttttgtctacacttatctacgtccaagatccctgcgatctccaacagaggacaaggttctggctgtcttctacaccaccctcactccaatgctcaaccccatcatctatagcctgaggaacaaggaggtgatgggggccctgacacgagtgagtcagagaatctgctctgggaaaatgtag

SEQ ID NO: 2 - protein, 312 aa, Homo sapiens
MENYNQTSTDFILLGFFPPSRIGLFLFILIVFIFLMALIGNLSMILLIFLDTHLHTPMYFLLSQLSLIDLNYISTIVPKMASDFLSGNKSISFTGCGIQSFFFSALGGAEALLLASMAYDRYIAICFPLHYPIRMSKRMCVLMITGSWIIGSINACAHTVYVLHIPYCQSRAINHFFCDVPAMVTLACMDTWVYEGTVFLSTTIFLVFPFIAISCSYGRVLLAVYHMKSAEGRKKAYLTCSTHLTVVTFYYAPFVYTYLRPRSLRSPTEDKVLAVFYTTLTPMLNPIIYSLRNKEVMGALTRVSQRICSGKM

SEQ ID NO: 3 - DNA, 2445 bp, Bos taurus
  CDS (1)..(1047)
atgaacgggaccgagggcccaaacttctacgtgcctttctccaacaagacgggcgtggtgcgcagccccttcgaggccccgcagtactacctggcggagccatggcagttctccatgctggccgcctacatgttcctgctgatcatgcttggcttccccatcaacttcctcacgctgtacgtcacagtccagcacaagaagctgcgcacacccctcaactacatcctgctcaacctggccgtggccgacctcttcatggtcttcgggggcttcaccaccaccctctacacctctctgcacggatacttcgtctttgggcccacgggctgcaacctggagggcttctttgccaccctgggcggtgaaattgcactgtggtccttggtggtcctggccatcgagcggtacgtggtggtgtgcaagcccatgagcaacttccgcttcggggagaaccacgccatcatgggcgtcgccttcacctgggtcatggctctggcctgtgccgcgccccccctcgtcggctggtccaggtacatcccggagggcatgcagtgctcgtgcgggattgactactacacgccccacgaggagaccaacaatgagtcgttcgtcatctacatgttcgtggtccacttcatcatccccctgattgtcatattcttctgctacgggcagctggtgttcaccgtcaaggaggcggctgcccagcagcaggagtcggccaccactcagaaggccgagaaggaggtcacccgcatggtgatcatcatggtcatcgctttcctaatctgctggctgccctacgctggggtggcgttctacatcttcacccatcagggctctgactttggccccatcttcatgaccatcccggctttctttgccaagacttctgccgtctacaaccccgtcatctacatcatgatgaacaagcagttccggaactgcatggtcaccactctctgctgtggcaagaacccgctgggtgacgacgaggcctccaccaccgtctccaagacagagaccagccaggtggcgcctgcctaagcccctccagggactccgtggccagctgcaggagtccctcagcccccaccccaccccagcctcagcagctccatcaggagccgcgcctgtcggaaccagctctcacaggctccctgagtgtaaacacaaagaccaaccaaccaaatgcaaaagaatcaacgagagaaacaggaggcgcctcacgtggcaggggcggcccgatctggagtcctgatttcccgggggcccgctgtagatccactccccccagctcatctctcagctacacaagagctcttgctctggaaaagtgtcccagcttagggataagtgagtagcacatgacggggcatgccgtaggtgcttattaataaatgctaggtggaggaaagaaggaatgaatggagagatgaacgggtcgggagggcataggcatcctcttacaacatgttagcagcagcagcagcagctcgcccttggctcatgaccttgagcagctgttttgtccttgggcctcactttcttcccccatacaatgggaattccaaatctctcctcacacgggctgctgggaagatcaaatgagattgtgtgtgtgtgcgtgcgtgcgtgctcgcttgtgtgagctctttgtaaatagtaaggagctggacagactgtagttaacattatgaataatatcaagtaatataagtaattcatctcctatgatcatctcctcttgatagcgaccactttgagactgggcaaggctctaagcatccagcctcgtcaggcttataaacattagacagatggcaaggtcagaccagcgccgggtggtgggccacagggaaggacggtcaaggaaatgcagagtgcaggcatcaggcctgagaagaaaacaaaaaccaaaaaaacaacatcagaggaccagagtctggggccagtgcagagcccccatgacgcgggccactccctcccagtgcaacccccagagagacaggtcttgctctcggcatctgaaaaaccactagctctcctgcccagcacccaggctgcagtatctctgggcccgtatggagcttctagaagttatgtttacctgcccacatttaacgaagagctgggtccccaacatcacctttgtctcaaaaagagcttaaaaaacaaaagcgtgggaaatccggctggacccaccttccccctgggaagttcacagatcacagattttagctcccttgctgggcaagccttcagcggctccagtccattctccactccggagagtccttgctgctgagaggctggctgggactctaggacatcagaatcgagccgcctcataactgcccctcctccactacataaccaaagcgggaagctctacctctccccagctctgcctggagacgaaggcaaattggggtattaaaagct

SEQ ID NO: 4 - protein, 348 aa, Bos taurus
MNGTEGPNFYVPFSNKTGVVRSPFEAPQYYLAEPWQFSMLAAYMFLLIMLGFPINFLTLYVTVQHKKLRTPLNYILLNLAVADLFMVFGGFTTTLYTSLHGYFVFGPTGCNLEGFFATLGGEIALWSLVVLAIERYVVVCKPMSNFRFGENHAIMGVAFTWVMALACAAPPLVGWSRYIPEGMQCSCGIDYYTPHEETNNESFVIYMFVVHFIIPLIVIFFCYGQLVFTVKEAAAQQQESATTQKAEKEVTRMVIIMVIAFLICWLPYAGVAFYIFTHQGSDFGPIFMTIPAFFAKTSAVYNPVIYIMMNKQFRNCMVTTLCCGKNPLGDDEASTTVSKTETSQVAPA